European Patent Application EP 4 506 458 A1, published February 12, 2025. Title: Fibrin lytic protein comprising an antibody that bind to fibrin and pharmaceutical formulation comprising the same. Applicant: RIN Institute Inc. Application JP. The sequence listing filed with the application follows.

SEQUENCE LISTING (63 sequences)

SEQ ID NO: 1 - protein, 656 aa, synthetic construct
  REGION 1..656: note = AMU1114 heavy chain
EVQLVQSGAEVKKPGESLKISCKGSGYSFTSYWMHWVRQMPGKGLEWIGAIYPGNSDTRYSPSFQGQVTISADKSISTAYLQWSSLKASDTAMYYCTRKAHYGNYGFAYWGQGTLVTVSSASTKGPSVFPLAPSSKSTSGGTAALGCLVKDYFPEPVTVSWNSGALTSGVHTFPAVLQSSGLYSLSSVVTVPSSSLGTQTYICNVNHKPSNTKVDKKVEPKSCGSGGGGSGGGGSGGSSSNELHQVPSNCDCLNGGTCVSNKYFSNIHWCNCPKKFGGQHCEIDKSKTCYEGNGHFYRGKASTDTMGRPCLPWNSATVLQQTYHAHRSDALQLGLGKHNYCRNPDNRRRPWCYVQVGLKPLVQECMVHDCADGGGPSSPPEELKFQCGQKTLRPRFKIIGGEFTTIENQPWFAAIYRRHRGGSVTYVCGGSLISPCWVISATHCFIDYPKKEDYIVYLGRSRLNSNTQGEMKFEVENLILHKDYSADTLAHHNDIALLKIRSKEGRCAQPSRTIQTICLPSMYNDPQFGTSCEITGFGKENSTDYLYPEQLKMTVVKLISHRECQQPHYYGSEVTTKMLCAADPQWKTDSCQGDSGGPLVCSLQGRMTLTGIVSWGRGCALKDKPGVYTRVSHFLPWIRSHTKEENGLALSAGGAS

SEQ ID NO: 2 - protein, 656 aa, synthetic construct
  REGION 1..656: note = AMU1114 F157D heavy chain
EVQLVQSGAEVKKPGESLKISCKGSGYSFTSYWMHWVRQMPGKGLEWIGAIYPGNSDTRYSPSFQGQVTISADKSISTAYLQWSSLKASDTAMYYCTRKAHYGNYGFAYWGQGTLVTVSSASTKGPSVFPLAPSSKSTSGGTAALGCLVKDYFPEPVTVSWNSGALTSGVHTFPAVLQSSGLYSLSSVVTVPSSSLGTQTYICNVNHKPSNTKVDKKVEPKSCGSGGGGSGGGGSGGSSSNELHQVPSNCDCLNGGTCVSNKYFSNIHWCNCPKKFGGQHCEIDKSKTCYEGNGHFYRGKASTDTMGRPCLPWNSATVLQQTYHAHRSDALQLGLGKHNYCRNPDNRRRPWCYVQVGLKPLVQECMVHDCADGGGPSSPPEELKFQCGQKTLRPRDKIIGGEFTTIENQPWFAAIYRRHRGGSVTYVCGGSLISPCWVISATHCFIDYPKKEDYIVYLGRSRLNSNTQGEMKFEVENLILHKDYSADTLAHHNDIALLKIRSKEGRCAQPSRTIQTICLPSMYNDPQFGTSCEITGFGKENSTDYLYPEQLKMTVVKLISHRECQQPHYYGSEVTTKMLCAADPQWKTDSCQGDSGGPLVCSLQGRMTLTGIVSWGRGCALKDKPGVYTRVSHFLPWIRSHTKEENGLALSAGGAS

SEQ ID NO: 3 - protein, 656 aa, synthetic construct
  REGION 1..656: note = AMU1114 F157E heavy chain
EVQLVQSGAEVKKPGESLKISCKGSGYSFTSYWMHWVRQMPGKGLEWIGAIYPGNSDTRYSPSFQGQVTISADKSISTAYLQWSSLKASDTAMYYCTRKAHYGNYGFAYWGQGTLVTVSSASTKGPSVFPLAPSSKSTSGGTAALGCLVKDYFPEPVTVSWNSGALTSGVHTFPAVLQSSGLYSLSSVVTVPSSSLGTQTYICNVNHKPSNTKVDKKVEPKSCGSGGGGSGGGGSGGSSSNELHQVPSNCDCLNGGTCVSNKYFSNIHWCNCPKKFGGQHCEIDKSKTCYEGNGHFYRGKASTDTMGRPCLPWNSATVLQQTYHAHRSDALQLGLGKHNYCRNPDNRRRPWCYVQVGLKPLVQECMVHDCADGGGPSSPPEELKFQCGQKTLRPREKIIGGEFTTIENQPWFAAIYRRHRGGSVTYVCGGSLISPCWVISATHCFIDYPKKEDYIVYLGRSRLNSNTQGEMKFEVENLILHKDYSADTLAHHNDIALLKIRSKEGRCAQPSRTIQTICLPSMYNDPQFGTSCEITGFGKENSTDYLYPEQLKMTVVKLISHRECQQPHYYGSEVTTKMLCAADPQWKTDSCQGDSGGPLVCSLQGRMTLTGIVSWGRGCALKDKPGVYTRVSHFLPWIRSHTKEENGLALSAGGAS

SEQ ID NO: 4 - protein, 656 aa, synthetic construct
  REGION 1..656: note = AMU1114 N22Y, N27S, H29R, W30R, Q40E, F157D heavy chain
EVQLVQSGAEVKKPGESLKISCKGSGYSFTSYWMHWVRQMPGKGLEWIGAIYPGNSDTRYSPSFQGQVTISADKSISTAYLQWSSLKASDTAMYYCTRKAHYGNYGFAYWGQGTLVTVSSASTKGPSVFPLAPSSKSTSGGTAALGCLVKDYFPEPVTVSWNSGALTSGVHTFPAVLQSSGLYSLSSVVTVPSSSLGTQTYICNVNHKPSNTKVDKKVEPKSCGSGGGGSGGGGSGGSSSNELHQVPSNCDCLNGGTCVSYKYFSSIRRCNCPKKFGGEHCEIDKSKTCYEGNGHFYRGKASTDTMGRPCLPWNSATVLQQTYHAHRSDALQLGLGKHNYCRNPDNRRRPWCYVQVGLKPLVQECMVHDCADGGGPSSPPEELKFQCGQKTLRPRDKIIGGEFTTIENQPWFAAIYRRHRGGSVTYVCGGSLISPCWVISATHCFIDYPKKEDYIVYLGRSRLNSNTQGEMKFEVENLILHKDYSADTLAHHNDIALLKIRSKEGRCAQPSRTIQTICLPSMYNDPQFGTSCEITGFGKENSTDYLYPEQLKMTVVKLISHRECQQPHYYGSEVTTKMLCAADPQWKTDSCQGDSGGPLVCSLQGRMTLTGIVSWGRGCALKDKPGVYTRVSHFLPWIRSHTKEENGLALSAGGAS

SEQ ID NO: 5 - protein, 656 aa, synthetic construct
  REGION 1..656: note = AMU1114 N22Y, N27S, H29R, W30R, Q40E, F157E heavy chain
EVQLVQSGAEVKKPGESLKISCKGSGYSFTSYWMHWVRQMPGKGLEWIGAIYPGNSDTRYSPSFQGQVTISADKSISTAYLQWSSLKASDTAMYYCTRKAHYGNYGFAYWGQGTLVTVSSASTKGPSVFPLAPSSKSTSGGTAALGCLVKDYFPEPVTVSWNSGALTSGVHTFPAVLQSSGLYSLSSVVTVPSSSLGTQTYICNVNHKPSNTKVDKKVEPKSCGSGGGGSGGGGSGGSSSNELHQVPSNCDCLNGGTCVSYKYFSSIRRCNCPKKFGGEHCEIDKSKTCYEGNGHFYRGKASTDTMGRPCLPWNSATVLQQTYHAHRSDALQLGLGKHNYCRNPDNRRRPWCYVQVGLKPLVQECMVHDCADGGGPSSPPEELKFQCGQKTLRPREKIIGGEFTTIENQPWFAAIYRRHRGGSVTYVCGGSLISPCWVISATHCFIDYPKKEDYIVYLGRSRLNSNTQGEMKFEVENLILHKDYSADTLAHHNDIALLKIRSKEGRCAQPSRTIQTICLPSMYNDPQFGTSCEITGFGKENSTDYLYPEQLKMTVVKLISHRECQQPHYYGSEVTTKMLCAADPQWKTDSCQGDSGGPLVCSLQGRMTLTGIVSWGRGCALKDKPGVYTRVSHFLPWIRSHTKEENGLALSAGGAS

SEQ ID NO: 6 - protein, 411 aa, Homo sapiens
SNELHQVPSNCDCLNGGTCVSNKYFSNIHWCNCPKKFGGQHCEIDKSKTCYEGNGHFYRGKASTDTMGRPCLPWNSATVLQQTYHAHRSDALQLGLGKHNYCRNPDNRRRPWCYVQVGLKPLVQECMVHDCADGKKPSSPPEELKFQCGQKTLRPRFKIIGGEFTTIENQPWFAAIYRRHRGGSVTYVCGGSLISPCWVISATHCFIDYPKKEDYIVYLGRSRLNSNTQGEMKFEVENLILHKDYSADTLAHHNDIALLKIRSKEGRCAQPSRTIQTICLPSMYNDPQFGTSCEITGFGKENSTDYLYPEQLKMTVVKLISHRECQQPHYYGSEVTTKMLCAADPQWKTDSCQGDSGGPLVCSLQGRMTLTGIVSWGRGCALKDKPGVYTRVSHFLPWIRSHTKEENGLAL

SEQ ID NO: 7 - protein, 411 aa, synthetic construct
  REGION 1..411: note = Pro-urokinase K135G, K136G
SNELHQVPSNCDCLNGGTCVSNKYFSNIHWCNCPKKFGGQHCEIDKSKTCYEGNGHFYRGKASTDTMGRPCLPWNSATVLQQTYHAHRSDALQLGLGKHNYCRNPDNRRRPWCYVQVGLKPLVQECMVHDCADGGGPSSPPEELKFQCGQKTLRPRFKIIGGEFTTIENQPWFAAIYRRHRGGSVTYVCGGSLISPCWVISATHCFIDYPKKEDYIVYLGRSRLNSNTQGEMKFEVENLILHKDYSADTLAHHNDIALLKIRSKEGRCAQPSRTIQTICLPSMYNDPQFGTSCEITGFGKENSTDYLYPEQLKMTVVKLISHRECQQPHYYGSEVTTKMLCAADPQWKTDSCQGDSGGPLVCSLQGRMTLTGIVSWGRGCALKDKPGVYTRVSHFLPWIRSHTKEENGLAL

SEQ ID NO: 8 - protein, 16 aa, synthetic construct
  REGION 1..16: note = Fibrinogen Bbeta 231-246
CNIPVVSGKECEEIIR

SEQ ID NO: 9 - protein, 15 aa, synthetic construct
  REGION 1..15: note = Fibrinogen gamma 232-246
KNWIQYKEGFGHLSP

SEQ ID NO: 10 - protein, 5 aa, synthetic construct
  REGION 1..5: note = Humanized 1101 HCDR1
SYWMH

SEQ ID NO: 11 - protein, 17 aa, synthetic construct
  REGION 1..17: note = Humanized 1101 HCDR2
AIYPGNSDTRYSPSFQG

SEQ ID NO: 12 - protein, 11 aa, synthetic construct
  REGION 1..11: note = Humanized 1101 HCDR3
KAHYGNYGFAY

SEQ ID NO: 13 - protein, 11 aa, synthetic construct
  REGION 1..11: note = Humanized 1101 LCDR1
RASQHINNWLA

SEQ ID NO: 14 - protein, 7 aa, synthetic construct
  REGION 1..7: note = Humanized 1101 LCDR2
GATSLQS

SEQ ID NO: 15 - protein, 9 aa, synthetic construct
  REGION 1..9: note = Humanized 1101 LCDR3
QQYWSTPLT

SEQ ID NO: 16 - protein, 242 aa, synthetic construct
  REGION 1..242: note = Humanized 1101 VH
MGSTAILALLLAVLQGVCAEVQLVQSGAEVKKPGESLKISCKGSGYSFTSYWMHWVRQMPGKGLEWIGAIYPGNSDTRYSPSFQGQVTISADKSISTAYLQWSSLKASDTAMYYCTRKAHYGNYGFAYWGQGTLVTVSSASTKGPSVFPLAPSSKSTSGGTAALGCLVKDYFPEPVTVSWNSGALTSGVHTFPAVLQSSGLYSLSSVVTVPSSSLGTQTYICNVNHKPSNTKVDKKVEPKSC

SEQ ID NO: 17 - protein, 236 aa, synthetic construct
  REGION 1..236: note = Humanized 1101 VL
MDMRVPAQLLGLLLLWLRGARCDIQMTQSPSSLSASVGDRVTITCRASQHINNWLAWYQQKPGKAPKLLISGATSLQSGVPSRFSGSGSGTDFTLTISSLQPEDFATYYCQQYWSTPLTFGQGTKVEIKRTVAAPSVFIFPPSDEQLKSGTASVVCLLNNFYPREAKVQWKVDNALQSGNSQESVTEQDSKDSTYSLSSTLTLSKADYEKHKVYACEVTHQGLSSPVTKSFNRGEC

SEQ ID NO: 18 - protein, 5 aa, synthetic construct
  REGION 1..5: note = Humanized 99 HCDR1
NYGMN

SEQ ID NO: 19 - protein, 17 aa, synthetic construct
  REGION 1..17: note = Humanized 99 HCDR2
WINTKIGEPTYAQKFQG

SEQ ID NO: 20 - protein, 4 aa, synthetic construct
  REGION 1..4: note = Humanized 99 HCDR3
LLDY

SEQ ID NO: 21 - protein, 17 aa, synthetic construct
  REGION 1..17: note = Humanized 99 LCDR1
RASQSVLYSSNQKNYLA

SEQ ID NO: 22 - protein, 7 aa, synthetic construct
  REGION 1..7: note = Humanized 99 LCDR2
WASSLQS

SEQ ID NO: 23 - protein, 8 aa, synthetic construct
  REGION 1..8: note = Humanized 99 LCDR3
HQYLSSYT

SEQ ID NO: 24 - protein, 113 aa, synthetic construct
  REGION 1..113: note = Humanized 99 VH
QVQLVQSGAEVKKPGASVKVSCKASGYTFTNYGMNWVRQAPGQGLEWMGWINTKIGEPTYAQKFQGRVTMTRDKSSSTAYMELSSLRSEDTAVYYCARLLDYWGQGTLVTVSS

SEQ ID NO: 25 - protein, 113 aa, synthetic construct
  REGION 1..113: note = Humanized 99 VL
DIQMTQSPSSLSASVGDRVTITCRASQSVLYSSNQKNYLAWYQQKPGKSPKLLIYWASSLQSGVPSRFSGSGSGTDFTLTISSLQPEDFATYYCHQYLSSYTFGQGTKVEIKR

SEQ ID NO: 26 - protein, 656 aa, synthetic construct
  REGION 1..656: note = AMU1114 N22Y, N27S, H29R, W30R, Q40E, F157D/E
  SITE 396: note = MISC_FEATURE - X = E or D
EVQLVQSGAEVKKPGESLKISCKGSGYSFTSYWMHWVRQMPGKGLEWIGAIYPGNSDTRYSPSFQGQVTISADKSISTAYLQWSSLKASDTAMYYCTRKAHYGNYGFAYWGQGTLVTVSSASTKGPSVFPLAPSSKSTSGGTAALGCLVKDYFPEPVTVSWNSGALTSGVHTFPAVLQSSGLYSLSSVVTVPSSSLGTQTYICNVNHKPSNTKVDKKVEPKSCGSGGGGSGGGGSGGSSSNELHQVPSNCDCLNGGTCVSYKYFSSIRRCNCPKKFGGEHCEIDKSKTCYEGNGHFYRGKASTDTMGRPCLPWNSATVLQQTYHAHRSDALQLGLGKHNYCRNPDNRRRPWCYVQVGLKPLVQECMVHDCADGGGPSSPPEELKFQCGQKTLRPRXKIIGGEFTTIENQPWFAAIYRRHRGGSVTYVCGGSLISPCWVISATHCFIDYPKKEDYIVYLGRSRLNSNTQGEMKFEVENLILHKDYSADTLAHHNDIALLKIRSKEGRCAQPSRTIQTICLPSMYNDPQFGTSCEITGFGKENSTDYLYPEQLKMTVVKLISHRECQQPHYYGSEVTTKMLCAADPQWKTDSCQGDSGGPLVCSLQGRMTLTGIVSWGRGCALKDKPGVYTRVSHFLPWIRSHTKEENGLALSAGGAS

SEQ ID NO: 27 - protein, 7 aa, synthetic construct
  REGION 1..7: note = 10-102 HCDR1
FTNYGMN

SEQ ID NO: 28 - protein, 12 aa, synthetic construct
  REGION 1..12: note = 10-102 HCDR2
WINTYTGEATYA

SEQ ID NO: 29 - protein, 4 aa, synthetic construct
  REGION 1..4: note = 10-102 HCDR3
LMDY

SEQ ID NO: 30 - protein, 11 aa, synthetic construct
  REGION 1..11: note = 10-102 LCDR1
KASQDINKYIA

SEQ ID NO: 31 - protein, 7 aa, synthetic construct
  REGION 1..7: note = 10-102 LCDR2
YTSTLQP

SEQ ID NO: 32 - protein, 8 aa, synthetic construct
  REGION 1..8: note = 10-102 LCDR3
LQYDNLTW

SEQ ID NO: 33 - protein, 10 aa, synthetic construct
  REGION 1..10: note = 34-105 HCDR1
KSVSTSGYSY

SEQ ID NO: 34 - skipped

SEQ ID NO: 35 - protein, 8 aa, synthetic construct
  REGION 1..8: note = 34-105 HCDR3
QHIRELTR

SEQ ID NO: 36 - protein, 8 aa, synthetic construct
  REGION 1..8: note = 34-105 LCDR1
GFTFSSYA

SEQ ID NO: 37 - protein, 7 aa, synthetic construct
  REGION 1..7: note = 34-105 LCDR2
ISSGGTT

SEQ ID NO: 38 - protein, 9 aa, synthetic construct
  REGION 1..9: note = 34-105 LCDR3
VRGGTIGAY

SEQ ID NO: 39 - protein, 10 aa, synthetic construct
  REGION 1..10: note = Fib-0355 HCDR1
QSVLYSSNQK

SEQ ID NO: 40 - protein, 8 aa, synthetic construct
  REGION 1..8: note = Fib-0355 HCDR2
YWASTRES

SEQ ID NO: 41 - protein, 4 aa, synthetic construct
  REGION 1..4: note = Fib-0355 HCDR3
YLSS

SEQ ID NO: 42 - protein, 7 aa, synthetic construct
  REGION 1..7: note = Fib-0355 LCDR1
YTFTNYG

SEQ ID NO: 43 - protein, 6 aa, synthetic construct
  REGION 1..6: note = Fib-0355 LCDR2
NTNTGE

SEQ ID NO: 44 - protein, 5 aa, synthetic construct
  REGION 1..5: note = Fib-0355 LCDR3
RLLDY

SEQ ID NO: 45 - protein, 5 aa, synthetic construct
  REGION 1..5: note = 99 HCDR1
NYGMN

SEQ ID NO: 46 - protein, 17 aa, synthetic construct
  REGION 1..17: note = 99 HCDR2
WINTKIGEPTYAEEFKG

SEQ ID NO: 47 - protein, 4 aa, synthetic construct
  REGION 1..4: note = 99 HCDR3
LLDY

SEQ ID NO: 48 - protein, 15 aa, synthetic construct
  REGION 1..15: note = 99 LCDR1
RASESVDSYGNSFMH

SEQ ID NO: 49 - protein, 7 aa, synthetic construct
  REGION 1..7: note = 99 LCDR2
RASNLES

SEQ ID NO: 50 - protein, 9 aa, synthetic construct
  REGION 1..9: note = 99 LCDR3
QQSNEDPRT

SEQ ID NO: 51 - protein, 5 aa, synthetic construct
  REGION 1..5: note = 1101 HCDR1
SYWMH

SEQ ID NO: 52 - protein, 17 aa, synthetic construct
  REGION 1..17: note = 1101 HCDR2
AIYPGNSDTRNNQKFKG

SEQ ID NO: 53 - protein, 11 aa, synthetic construct
  REGION 1..11: note = 1101 HCDR3
KAHYGNYGFAY

SEQ ID NO: 54 - protein, 11 aa, synthetic construct
  REGION 1..11: note = 1101 LCDR1
KASDHINNWLA

SEQ ID NO: 55 - protein, 7 aa, synthetic construct
  REGION 1..7: note = 1101 LCDR2
GATSLET

SEQ ID NO: 56 - protein, 9 aa, synthetic construct
  REGION 1..9: note = 1101 LCDR3
QQYWSTPLT

SEQ ID NO: 57 - protein, 5 aa, synthetic construct
  REGION 1..5: note = 0211 HCDR1
SYAMS

SEQ ID NO: 58 - protein, 16 aa, synthetic construct
  REGION 1..16: note = 0211 HCDR2
AISSGGTTYYPDSVKG

SEQ ID NO: 59 - protein, 8 aa, synthetic construct
  REGION 1..8: note = 0211 HCDR3
GGTIGAYW

SEQ ID NO: 60 - protein, 17 aa, synthetic construct
  REGION 1..17: note = 0211 LCDR1
KSSQSVLYSSNQKNYLA

SEQ ID NO: 61 - protein, 7 aa, synthetic construct
  REGION 1..7: note = 0211 LCDR2
WASTRES

SEQ ID NO: 62 - protein, 8 aa, synthetic construct
  REGION 1..8: note = 0211 LCDR3
HQYLSSWT

SEQ ID NO: 63 - protein, 651 aa, synthetic construct
EVQLVQSGAEVKKPGESLKISCKGSGYSFTSYWMHWVRQMPGKGLEWIGAIYPGNSDTRYSPSFQGQVTISADKSISTAYLQWSSLKASDTAMYYCTRKAHYGNYGFAYWGQGTLVTVSSASTKGPSVFPLAPSSKSTSGGTAALGCLVKDYFPEPVTVSWNSGALTSGVHTFPAVLQSSGLYSLSSVVTVPSSSLGTQTYICNVNHKPSNTKVDKKVEPKSCGSGGGGSGGGGSGGSSSNELHQVPSNCDCLNGGTCVSGGHWCNCPKKFGGQHCEIDKSKTCYEGNGHFYRGKASTDTMGRPCLPWNSATVLQQTYHAHRSDALQLGLGKHNYCRNPDNRRRPWCYVQVGLKPLVQECMVHDCADGGGPSSPPEELKFQCGQKTLRPREKIIGGEFTTIENQPWFAAIYRRHRGGSVTYVCGGSLISPCWVISATHCFIDYPKKEDYIVYLGRSRLNSNTQGEMKFEVENLILHKDYSADTLAHHNDIALLKIRSKEGRCAQPSRTIQTICLPSMYNDPQFGTSCEITGFGKENSTDYLYPEQLKMTVVKLISHRECQQPHYYGSEVTTKMLCAADPQWKTDSCQGDSGGPLVCSLQGRMTLTGIVSWGRGCALKDKPGVYTRVSHFLPWIRSHTKEENGLALSAGGAS